European Patent Application EP 4 631 969 A1, published October 15, 2025. Title: Peptide for cartilage regeneration and uses thereof. Applicant: CAREGEN CO., LTD. The sequence listing filed with the application follows.

SEQUENCE LISTING (16 sequences)

SEQ ID NO: 1 - protein, 12 aa, synthetic construct
STGALSTSFTEE

SEQ ID NO: 2 - protein, 5 aa, synthetic construct
HHEQF

SEQ ID NO: 3 - DNA, 23 bp, synthetic construct
  source 1..23: mol_type = other DNA
ctatctggacgaagcagctggca

SEQ ID NO: 4 - DNA, 22 bp, synthetic construct
  source 1..22: mol_type = other DNA
atgggtgcaatgtcaatgatgg

SEQ ID NO: 5 - DNA, 20 bp, synthetic construct
  source 1..20: mol_type = other DNA
aactcagggcaggaggatgt

SEQ ID NO: 6 - DNA, 20 bp, synthetic construct
  source 1..20: mol_type = other DNA
tgtccttttggtcgtcgttc

SEQ ID NO: 7 - DNA, 20 bp, synthetic construct
  source 1..20: mol_type = other DNA
ccagcccgaacttgtaaaga

SEQ ID NO: 8 - DNA, 20 bp, synthetic construct
  source 1..20: mol_type = other DNA
tggacgcacaaccatcatac

SEQ ID NO: 9 - DNA, 20 bp, synthetic construct
  source 1..20: mol_type = other DNA
tgagtcctcaagcctcctgt

SEQ ID NO: 10 - DNA, 20 bp, synthetic construct
  source 1..20: mol_type = other DNA
gtgccagatcatcaccacac

SEQ ID NO: 11 - DNA, 20 bp, synthetic construct
  source 1..20: mol_type = other DNA
gcaggctatgagcagtgtga

SEQ ID NO: 12 - DNA, 20 bp, synthetic construct
  source 1..20: mol_type = other DNA
gcatacctcggaagcagaag

SEQ ID NO: 13 - DNA, 20 bp, synthetic construct
  source 1..20: mol_type = other DNA
accacagtccatgccatcac

SEQ ID NO: 14 - DNA, 20 bp, synthetic construct
  source 1..20: mol_type = other DNA
tccaccaccctgttgctgta

SEQ ID NO: 15 - DNA, 20 bp, synthetic construct
  source 1..20: mol_type = other DNA
gcggaggaagtcggtgaaga

SEQ ID NO: 16 - DNA, 20 bp, synthetic construct
  source 1..20: mol_type = other DNA
ccctctcgcttcaggtcagc